European Patent Specification EP 3 277 713 B1, published September 10, 2025. Title: Polypeptides. Applicant: VHsquared Limited. The sequence listing filed with the application follows.

SEQUENCE LISTING (35 sequences)

SEQ ID NO: 1 - protein, 115 aa, Artificial Sequence
  Polypeptide sequence of anti-TNF-alpha ICVD Q65B1
EVQLVESGGGLVQPGGSLKLSCAASGFDFSSHWMYWVRQAPGKELEWLSEINTNGLITKYGDSVKGRFTVSRNNAANKMYLELTRLEPEDTALYYCARNQKGLNKGQGTQVTVSS

SEQ ID NO: 2 - protein, 115 aa, Artificial Sequence
  Polypeptide sequence of anti-TNF-alpha ICVD ID8F-EV (ID32F)
EVQLVESGGGLVQPGGSLKLSCAASGFDFSSHWMYWVRQAPGKELEWLSEINTNGLITHYGDSVKGRFTVSRNNAANKMYLELTRLEPEDTALYYCARNQKGLNKGQGTQVTVSS

SEQ ID NO: 3 - protein, 115 aa, Artificial Sequence
  Polypeptide sequence of anti-TNF-alpha ICVD ID43F
EVQLVESGGGLVQPGGSLKLSCAASGFDFSSHWMYWVRQAPGKELEWLSEINTNGLITAYGDSVKGRFTVSRNNAANKMYLELTRLEPEDTALYYCARNQKGLNKGQGTQVTVSS

SEQ ID NO: 4 - protein, 115 aa, Artificial Sequence
  Polypeptide sequence of anti-TNF-alpha ICVD ID44F
EVQLVESGGGLVQPGGSLKLSCAASGFDFSSHWMYWVRQAPGKELEWLSEINTNGLITQYGDSVKGRFTVSRNNAANKMYLELTRLEPEDTALYYCARNQKGLNKGQGTQVTVSS

SEQ ID NO: 5 - protein, 115 aa, Artificial Sequence
  Polypeptide sequence of anti-TNF-alpha ICVD ID34F
EVQLVESGGGLVQPGGSLKLSCAASGFDFSSHWMYWVRQAPGKELEWLSEINTNGLITHYGDSVKGRFTVSRNNAANKMYLELTRLEPEDTALYYCARNQHGLNKGQGTQVTVSS

SEQ ID NO: 6 - protein, 122 aa, Artificial Sequence
  Polypeptide sequence of anti-TcdB ICVD B10F1
QVQLQESGGGLVQAGGSLRLSCAASGRTFSSYYMGWFRQAPGKEREFVAAINGSGGNRISADSVKGRFTISRDNAKNTVYLQLNSLKPEDTAVYYCAASLTYYGRSARYDYWGQGTQVTVSS

SEQ ID NO: 7 - protein, 124 aa, Artificial Sequence
  Polypeptide sequence of anti-TcdB ICVD Q31B1
EVQLVESGGGLVQAGDSLRLSCAASGRTLSSYTMGWFRQAPEKEREFVAGSSRDGRTNYYANSVKGRFTISRDNAKNTVYLQMNSLKPEDTAVYYCAAHTTSGVPVRERSYAYWGQGTQVTVSS

SEQ ID NO: 8 - protein, 122 aa, Artificial Sequence
  Polypeptide sequence of anti-TcdB ICVD ID1B
DVQLQESGGGLVQAGGSLRLSCAASGATFSSYYMGWFRQAPGKEREFVAAINGSGGNRISADSVKGRFTISRDNAKNTVYLQLNSLKPEDTAVYYCAASLTYYGRSARYDYWGQGTQVTVSS

SEQ ID NO: 9 - protein, 124 aa, Artificial Sequence
  Polypeptide sequence of anti-TcdB ICVD ID2B
DVQLQESGGGLVQAGDSLRLSCAASGATLSSYTMGWFRQAPEKEREFVAGSSRDGRTNYYANSVKGRFTISRDNAKNTVYLQMNSLKPEDTAVYYCAAHTTSGVPVRERSYAYWGQGTQVTVSS

SEQ ID NO: 10 - protein, 124 aa, Artificial Sequence
  Polypeptide sequence of anti-TcdB ICVD ID20B
DVQLQESGGGLVQAGDSLRLSCAASGATLSSYTIGWFRQAPEKEREFVAGSSHDGHTNYYANSVKGRFTISRDNAKNTVYLQMNSLKPEDTAVYYCAAHTTSGVPVRERSYAYWGQGTQVTVSS

SEQ ID NO: 11 - protein, 124 aa, Artificial Sequence
  Polypeptide sequence of anti-TcdB ICVD ID21B
DVQLQESGGGLVQAGDSLRLSCAASGATLSSYTIGWFRQAPEKEREFVAGSSRDGRTNYYANSVKGRFTISRDNAKNTVYLQMNSLKPEDTAVYYCAAHTTSGVPVHERSYAYWGQGTQVTVSS

SEQ ID NO: 12 - protein, 124 aa, Artificial Sequence
  Polypeptide sequence of anti-TcdB ICVD ID22B
DVQLQESGGGLVQAGDSLRLSCAASGATLSSYTIGWFRQAPEKEREFVAGSSRDGRTNYYANSVKGRFTISRDNAKNTVYLQMNSLKPEDTAVYYCAAHTTSGVPVREHSYAYWGQGTQVTVSS

SEQ ID NO: 13 - protein, 122 aa, Artificial Sequence
  Polypeptide sequence of anti-TcdB ICVD ID24B
DVQLQESGGGLVQAGGSLRLSCAASGATFSSYYIGWFRQAPGKEREFVAAINGSGGNHISADSVKGRFTISRDNAKNTVYLQLNSLKPEDTAVYYCAASLTYYGRSARYDYWGQGTQVTVSS

SEQ ID NO: 14 - protein, 122 aa, Artificial Sequence
  Polypeptide sequence of anti-TcdB ICVD ID25B
DVQLQESGGGLVQAGGSLRLSCAASGATFSSYYIGWFRQAPGKEREFVAAINGSGGNRISADSVKGRFTISRDNAKNTVYLQLNSLKPEDTAVYYCAASLTYYGRSAHYDYWGQGTQVTVSS

SEQ ID NO: 15 - protein, 122 aa, Artificial Sequence
  Polypeptide sequence of anti-TcdB ICVD ID27B
DVQLQESGGGLVQAGGSLRLSCAASGATFSSYYIGWFRQAPGKEREFVAAINGSGGNRISADSVKGRFTISRDNAKNTVYLQLNSLKPEDTAVYYCAASLTYYGHSARYDYWGQGTQVTVSS

SEQ ID NO: 16 - protein, 266 aa, Artificial Sequence
  Polypeptide sequence of anti-TcdB construct ID41B
DVQLQESGGGLVQAGDSLRLSCAASGATLSSYTMGWFRQAPEKEREFVAGSSRDGRTNYYANSVKGRFTISRDNAKNTVYLQMNSLKPEDTAVYYCAAHTTSGVPVHERSYAYWGQGTQVTVSSGGGGSGGGGSGGGGSGGGGSDVQLQESGGGLVQAGGSLRLSCAASGATFSSYYMGWFRQAPGKEREFVAAINGSGGNRISADSVKGRFTISRDNAKNTVYLQLNSLKPEDTAVYYCAASLTYYGHSARYDYWGQGTQVTVSS

SEQ ID NO: 17 - protein, 266 aa, Artificial Sequence
  Polypeptide sequence of anti-TcdB construct ID43B
DVQLQESGGGLVQAGDSLRLSCAASGATLSSYTMGWFRQAPEKEREFVAGSSRDGRTNYYANSVKGRFTISRDNAKNTVYLQMNSLKPEDTAVYYCAAHTTSGVPVHERSYAYWGQGTQVTVSSGGGGSGGGGSGGGGSGGGGSDVQLQESGGGLVQAGGSLRLSCAASGATFSSYYMGWFRQAPGKEREFVAAINGSGGNRISADSVKGRFTISRDNAKNTVYLQLNSLKPEDTAVYYCAASLTYYGHSAHYDYWGQGTQVTVSS

SEQ ID NO: 18 - protein, 124 aa, Artificial Sequence
  Polypeptide sequence of anti-TcdB ICVD ID45B
EVQLVESGGGLVQAGDSLRLSCAASGATLSSYTMGWFRQAPEKEREFVAGSSRDGRTNYYANSVKGRFTISRDNAKNTVYLQMNSLKPEDTAVYYCAAHTTSGVPVRERSYAYWGQGTQVTVSS

SEQ ID NO: 19 - protein, 124 aa, Artificial Sequence
  Polypeptide sequence of anti-TcdB ICVD ID46B
EVQLVESGGGLVQAGDSLRLSCAASGATLSSYTMGWFRQAPEKEREFVAGSSRDGRTNYYANSVKGRFTISRDNAKNTVYLQMNSLKPEDTAVYYCAAHTTSGVPVHERSYAYWGQGTQVTVSS

SEQ ID NO: 20 - protein, 124 aa, Artificial Sequence
  Polypeptide sequence of anti-TcdB ICVD ID47B
EVQLVESGGGLVQAGDSLRLSCAASGATLSSYTMGWFRQAPEKEREFVAGSSRDGRTNYYANSVKGRFTISRDNAKNTVYLQMNSLKPEDTAVYYCAAHTTSGVPVAERSYAYWGQGTQVTVSS

SEQ ID NO: 21 - protein, 124 aa, Artificial Sequence
  Polypeptide sequence of anti-TcdB ICVD ID48B
EVQLVESGGGLVQAGDSLRLSCAASGATLSSYTMGWFRQAPEKEREFVAGSSRDGRTNYYANSVKGRFTISRDNAKNTVYLQMNSLKPEDTAVYYCAAHTTSGVPVQERSYAYWGQGTQVTVSS

SEQ ID NO: 22 - protein, 124 aa, Artificial Sequence
  Polypeptide sequence of anti-TcdB ICVD ID49B
EVQLVESGGGLVQAGDSLRLSCAASGATLSSYTMGWFRQAPEKEREFVAGSSRDGRTNYYANSVKGRFTISRDNAKNTVYLQMNSLKPEDTAVYYCAAHTTSGVPVFERSYAYWGQGTQVTVSS

SEQ ID NO: 23 - protein, 124 aa, Artificial Sequence
  Polypeptide sequence of anti-TcdB ICVD ID50B
EVQLVESGGGLVQAGDSLRLSCAASGATLSSYTMGWFRQAPEKEREFVAGSSRDGRTNYYANSVKGRFTISRDNAKNTVYLQMNSLKPEDTAVYYCAAHTTSGVPVWERSYAYWGQGTQVTVSS

SEQ ID NO: 24 - protein, 257 aa, Artificial Sequence
  Polypeptide sequence of anti-TcdA construct ID17A
DVQLQESGGGLVQAGGSLRLSCAASGATSDVYAMGWFRQVPGKEREFVATINRSGSDSYYADSVKGRFTISRDNAKNTVYLQMNSLKPEETAVYYCAASRSDCIGYGCRRVSQDYWGQGTQVTVSSGGGGSGGGGSGGGGSGGGGSDVQLQESGGGLVQAGGSLRLSCVISGMDFSHKPAGWFRQAPGKEREFVASITTRASTHYADSVKGRFTISRDNAKNTVYLEMNSLKPEDTAVYYCNSEYYWGQGTQVTVSS

SEQ ID NO: 25 - protein, 257 aa, Artificial Sequence
  Polypeptide sequence of anti-TcdA construct ID29A
DVQLQESGGGLVQAGGSLRLSCAASGATSDVYAMGWFRQVPGKEREFVATINRSGSDSYYADSVKGRFTISRDNAKNTVYLQMNSLKPEETAVYYCAASRSDCIGYGCHRVSQDYWGQGTQVTVSSGGGGSGGGGSGGGGSGGGGSDVQLQESGGGLVQAGGSLRLSCVISGMDFSHKPAGWFRQAPGKEREFVASITTRASTHYADSVKGRFTISRDNAKNTVYLEMNSLKPEDTAVYYCNSEYYWGQGTQVTVSS

SEQ ID NO: 26 - protein, 15 aa, Artificial Sequence
  Example CDR A
ARNECDQGHILKMFP

SEQ ID NO: 27 - protein, 5 aa, Artificial Sequence
  First third of Example CDR A
ARNEC

SEQ ID NO: 28 - protein, 5 aa, Artificial Sequence
  Second third of Example CDR A
DQGHI

SEQ ID NO: 29 - protein, 5 aa, Artificial Sequence
  Third third of Example CDR A
LKMFP

SEQ ID NO: 30 - protein, 8 aa, Artificial Sequence
  Example CDR B
ARNECDQG

SEQ ID NO: 31 - protein, 4 aa, Artificial Sequence
  Second third of Example CDR B
NECD

SEQ ID NO: 32 - protein, 120 aa, Artificial Sequence
  Polypeptide sequence of anti-IL6R ICVD 7F6
EVQLVESGGGLVQAGGSTRLTCLASGSISSINVIGWYRQAPGKQRELVAMIGRGEGANYGDFAKGRFTISRDNSKNTVYLQMNSLKPEDTAVYYCYADYEDRDSPFNGSWGQGTQVTVSS

SEQ ID NO: 33 - protein, 120 aa, Artificial Sequence
  Polypeptide sequence of anti-IL6R ICVD ID-3V
EVQLVESGGGLVQAGGSTRLTCLASGSISSINVIGWYRQAPGKQRELVAMIGRGEGANYGDFAKGRFTISRDNSKNTVYLQMNSLKPEDTAVYYCYADYEDHDSPFNGSWGQGTQVTVSS

SEQ ID NO: 34 - protein, 123 aa, Artificial Sequence
  Polypeptide sequence of anti-IL6R ICVD 5G9
EVQLVESGGGLVQAGGSTRLTCKASGSIFNINSINVMAWYRQAPGKQRELVAIIGKGGGTNYADFVKGRFTISRDAAKNTVNLQMNSLKPEDTAVYYCYADYEDRDSPFNASWGQGTQVTVSS

SEQ ID NO: 35 - protein, 123 aa, Artificial Sequence
  Polypeptide sequence of anti-IL6R ICVD ID-54V
EVQLVESGGGLVQAGGSTRLTCKASGSIFNINSINVMAWYRQAPGKQRELVAIIGKGGGTNYADFVKGRFTISRDAAKNTVNLQMNSLKPEDTAVYYCYADYEDHDSPFNASWGQGTQVTVSS